European Patent Application EP 4 234 720 A1, published August 30, 2023. Title: EPIGENETIC BIOMARKERS FOR THE DIAGNOSIS OF THYROID CANCER. Applicant: Consejo Superior de Investigaciones Cientificas (CSIC) FUNDACION PARA LA INVESTIGACION E INNOVACION BIOSANITARIA PRINCIPADO DE ASTURIAS (FINBA). The sequence listing filed with the application follows.

SEQUENCE LISTING (9 sequences)

SEQ ID NO: 1 - DNA, 25 bp, Artificial Sequence
  Forward primer chr13:97858492- 97858493
aagattgaaagaattgggtatggaa

SEQ ID NO: 2 - DNA, 27 bp, Artificial Sequence
  Reverse primer chr13:97858492- 97858493
  misc_binding (1)..(1): Biotin
taacccaacaaaatttactcccctatc

SEQ ID NO: 3 - DNA, 18 bp, Artificial Sequence
  Sequencing primer chr13:97858492- 97858493
cctcaaaaaacaaaccac

SEQ ID NO: 4 - DNA, 23 bp, Artificial Sequence
  Forward primer chr14:74957673-74957674
  misc_binding (1)..(1): Biotin
aaggtgggtgtagagtggaatat

SEQ ID NO: 5 - DNA, 28 bp, Artificial Sequence
  Reverse primer chr14:74957673-74957674
ataactcattccatcctcacaaactatc

SEQ ID NO: 6 - DNA, 24 bp, Artificial Sequence
  Sequencing primer chr14:74957673-74957674
ggaaatttaaagtggtttataaag

SEQ ID NO: 7 - DNA, 23 bp, Artificial Sequence
  Forward primer chr20:5672830-5672831
tgaagggagtgagggtttattag

SEQ ID NO: 8 - DNA, 30 bp, Artificial Sequence
  Reverse primer chr20:5672830-5672831
  misc_binding (1)..(1): Biotin
ctaaccacttcacaaaactcttttacttat

SEQ ID NO: 9 - DNA, 18 bp, Artificial Sequence
  Sequencing primer chr20:5672830-5672831
agattagagtaggtgttg